European Patent Specification EP 4 463 867 B1, published May 20, 2026. Title: Synthetic promoters generated based on genomic DNA sequences. Applicant: Danmarks Tekniske Universitet. The sequence listing filed with the application follows.

SEQUENCE LISTING (8 sequences)

SEQ ID NO: 1 - DNA, 683 bp, synthetic construct
  misc_feature 1..683: note = Synthetic constitutive promoter
  misc_feature 1..683: note = Synthetic constitutive promoter BBa_K3046001|PLEAPglaA_2|low
  source 1..683: mol_type = other DNA
cgtccagctccataagctgggtatcccactccgattgactatgattcatgctagctggaagtcaatctcgggtagtgttatactggacgtatctcggcatgacaggcgataagtggaaggatgcatgcacggaatgcaaagcataggattgatctacggaaatgggactcccgatttgtcgccaaacgatgcaccgtggcccacgcatgacccctacttttgcgagttgcttgatacctagtcggacccaaaaaacatccgagttcacagcctgtgcttagtccgaaggcctcagatggcgaatgtacgtggagaatatggttgaatcttaagaacgtgaggttaatggttggaccacgtgggctcacctcacgcgcagctgcggagccgctagaatcgtcgtgttgattgtaaacttacatcccgccattagactaaagtcggcattggtaatgtcagggaaaaccgtgtgtcggataatgcccgcgatcctatgcgctttctactcggtatcgcgtgagcttgcactgaacgatcagcacacaaaccctgtgcactcgctatacactaacaacaaagttttaaaagagctcgctttcgcaatgcgcagagacactgagtgcagctgcctccttcttcagtctccacctctcctttatattatatttgcgcagtcgcctcgc

SEQ ID NO: 2 - DNA, 842 bp, synthetic construct
  misc_feature 1..842: note = Synthetic constitutive promoter
  misc_feature 1..842: note = Synthetic constitutive promoter BBa_K3046002|PLEAPsonB_1|low
  source 1..842: mol_type = other DNA
ttttttgttgtccaatgtagtttgggctgttccttcacatgacagcagtgttgggctagagagagaagaggatctgattgcgagaatccaggatgcgtcgacggcgacaggcgacagtccctcatccgtactgttactctgatacgtgcctcggaatcctaaggggcttgaatcaacagaatcagcagacaagatgatcgcagcttctaggatgcagtcagctgaccggatctggctccgtaattcaggcttcggaggggcatcaacggcacgtgacttaatgcggcggtaccacacccggtggtccctcggaaaaccctccagtaccagcggtaccgttccagatctgaccttaccggctgttccgcagccgtaagcgaggcaggcagcggtaacactacccgtccttcgctctctctctcccttctcttctcttcatctctccgctttttcccttcaccgtcgcgcgtcctcttctctttcccctcacctcttcatctttttctctctcgctttcgacccttcctttcggacttgttcacatcctagctttgacggtgacttcccgtctgtagctggtgtggccctttttttttgcttttctagatcccttcgcaaaacaaaacaccttttctctgtttttctgcgcgtcgagatctctcttcgcgagccactctttcgcctctactttgtgctagcgcactgcgatcgatcttttcgcctactgttatttcttgatacatcagctttagttatcgtcgttttacgagctttccaacttttcggtcgccgccctccttcgaacggatgaatccataatccgcagcaacaacaaacagcaa

SEQ ID NO: 3 - DNA, 926 bp, synthetic construct
  misc_feature 1..926: note = Synthetic constitutive promoter
  misc_feature 1..926: note = Synthetic constitutive promoter BBa_K3046003|PLEAPgpdA_1|high
  source 1..926: mol_type = other DNA
caccatggtaagcgcgtgatcgctcgtgtgcctaaccggtgactctttctggagtgcggagagaacgagggacgcctagagagaagcctaagcgatccagccagtgccggcaaagaggaggggcagtggatcatcgttattccgtgccgggctcacgggccgaaagcggaaaggccggagtgcccctcatttttggtgggaagcgtgggatggtggtgttccattacatcatcccttcctttggggcaattcccctcctccgcggcagtatgcgggtaggaacgtaaaaaccgggggatagacccgtcgtcccgagatcgccttcccaataacctaggtagaacagcccaattgattccgaaaagctggcaaaagattcacgagatggtaggagtgagtacccggcgtgatggatatggagcacgctcattggcccatccggcagctgccgaggggaggcaggagtcccaaatatcgtgagtctcctgctttgcccggtgtatgaaaccggaaagggctgctggggagctggggagcggcgcaagccgggaacacaagctgacaattgacccatttcctgcacattggcagagcttgcggtagcttttgccccgtctgtccgcccggtgtgcggactggcgcgaggaagaggtgacctggtcgttgcgtcaatccattctgtcgctatcctttttctacttcccctcccccgccgctgaacttttcttctctcttcttctctctttctctcttcatcatcatctcccttctatctccatcttcttttcatccaattaccttaaagtaagtcctctcccccccatccttcctcttcatcttcttcatccccttgtactttccttcctcttccctccctcacgaagctttactaacagctaccccgcccccaacagacacatctaaac

SEQ ID NO: 4 - DNA, 926 bp, synthetic construct
  misc_feature 1..926: note = Synthetic constitutive promoter
  misc_feature 1..926: note = Synthetic constitutive promoter BBa_K3046004|PLEAPgpdA_2|low
  source 1..926: mol_type = other DNA
caacaatataaaatcgtgatcactcctatggacggccggtgactctttctggagcaccgagagaacatggggggccagaggtcgtccgcctgggggactttcagcgacaccaacgaagaggagcaggggattatcattcctacagaccggtggaaccggccgaaagcggcaaggccggggtgcccctcgttgccttatgcaagtaggggccgtttgtcttctgttacatcatccactccccgacttgcaccccccacttccgcaatagttatcgccgcgaattgggaaacccgaggaaagaacctgtcttgccgacatggagatgctcataacccaggtacatgaggccaagtgattccgacattctggcaaaaggttcacgagttagtatcagtgtgtacccggcgtgctagatgcgaggcgcggttattggcccagccggtagcagccgaagacagacaggtctgccaaatatcgtgaatctcctgctttgcccggtgtatgaaaccggaagaggctgcttaggaacggcggggcggcgtaagtcgggaaactaagctgacatttaacccttttcccgtacactggaagcgcttcttgtggcttttgccccgtctgtccgcccggtgtgttaacgggcgcaaggtgttagtgaccaggtcgttgcgtcaatcaattgccttgctatcctttttcttcttccgctcccccaccgtcggacttttctttcctcttttactctctcttcctcttcatcatcctctatcctctatcttcttctttttatcatccttatcactaaaagtgagtccccctcggtgaattgaccttttcgaactcctccatcatagccgcttccccttctcccactctccgtcacgtagctctgctaacagctaccccgccctaaacagacacatccacac

SEQ ID NO: 5 - DNA, 986 bp, synthetic construct
  misc_feature 1..986: note = Synthetic constitutive promoter
  misc_feature 1..986: note = Synthetic constitutive promoter BBa_K3046005|PLEAPmstA_1|high
  source 1..986: mol_type = other DNA
gttgatcagggtccaagaagcctatttcgtgatcggaaacccaaaagggaggccctaaccggatccggctagtgctgggacccgagattgtggggaatccatcccgggcgaacacgtggtaggctgaattttccgacccctgtccattcccgccaatcagggcgggtcctactcgggcttgtccggctattaccagcctagccagcccgactgtcagtccggcgctgacccgagcctctgtttggccagatccccctggcttgtcccaaccacagcgaactagccaaggacataagtccgctatgccaagtggctggggttagcttgagtgtgccctcctagactgtcgtcgcccactccggggttggataccttatagtcagccggaggaaggtagtacagtacacccgcccctagccatgccaatgtaacctataaactgaaatccggctcctcagccccatgattggccggcaatcatttttctcctgaagtaggcaatcctaatcaggactggttgtaattttggcccctgtgcgtcccctcggccagcccccaggacgatggcaaatcgaggttcacggcattggctggtaaatcgtcccatctagtcggggcaagacgagaaaaaaaacaggtcaaatgaaaatggagtcatgaactcatggagccgagtgttaggtgcattccccgtgggcaattccccggacccggttctgggccgattcacgccatggggaaaccgcgagtctatgcagctccgtttctccctcaacggattataaaaccccctgcttccccccccctcttttctcccctgcttctctttccctcttcttcttcgatcttcctccttaccttcactctccttccctttttggttgccatagcggcttctccccccctccccagccctccctttccttctctctcttattctcttactttacagagcatcacgcagtctcctcctcgacatcagtcac

SEQ ID NO: 6 - DNA, 933 bp, synthetic construct
  misc_feature 1..933: note = Synthetic constitutive promoter
  misc_feature 1..933: note = Synthetic constitutive promoter BBa_K3046006|PLEAPunk_1:An07g08210|low
  source 1..933: mol_type = other DNA
attgatgaggggacgaatgccaaggctggagcataatttatttacatattgagattgatgactatatcctttcttagaacggactgaatatcattggagcctatgctgagttacacttaaatagttatcctgcattatggaaaaacaatgtcgatggttgggtaaatagttatgagcaggttagcaatcatttctctgatgaacttgtctgcttagatctgtgagtggatcttgttatccgttgatcaatcgaacatactcagggaatcaaccacaccgtacatactattctactaatcctagtaactcagcaataacgattatataaattatctcttactccgtaatcagaagtgccatcgtggcacctgagtggatctgtggctggaatgatgatcgacgtcactagataaggaagtgtggcgcagtcacctgaccgcgcccaccatacccgatcgggagatttgttttcggggaggctgggaaactcgcttccccctccgatttacttcccctcccccccccgcttccctatcgctgtctctctttctttcttttttttattgtcgttgcagcatccatctcttttctcgtttcaatccatctgcacgtcaatttttttctttttctttctttttgattttccctttcttttctcctgtttctgatctcgaatcaggacctctccgggacggagatcctcccgtttctatatcaacccatttttcccgcccaattcctcccgttaccatagggctatgcagcttctcccttgaatgagcattccatcccagtcaaaaccacacaactactattgcacatcactcggccgatttactgcttcggttggtgaagcaggtatgcggccaattgaagtcgagactcccctatttccgttggttttcgcattcttgtccacggaacggcaccagt

SEQ ID NO: 7 - DNA, 973 bp, synthetic construct
  misc_feature 1..973: note = Synthetic constitutive promoter
  misc_feature 1..973: note = Synthetic constitutive promoter BBa_K3046007|PLEAPgfaA_1|medium
  source 1..973: mol_type = other DNA
ttcacaccagaggcaaaatctactgtgggatactactcaagtacaaagaggggctccctcacgatttagaggtctgtatctgcgagattctatgattaagggtagcaacatgaataagacgcatagcaactaccgacagggtgctaataactttatttgtcgccaataacttgattttttgcattttccacttgtagatgactacatgcgtatctataaataatagatagggggggagaagtttctacctagaactaaaaatattattagaaacctttgggtgtgttatttttagaaactttcgccatcgtctatactcgaacaaaatccatggagacagggagaaatattgactggtagctaataatagtcggtatgttatttttgacctcccaagtggggatgattacctctttaattcttagtagatatagttagcactctattttccatgccatgggatggtcggttgtcctgaaccgagtcacgagtgagacataccaatagactgtgtgaggcgcagagtgggcttattggccacttcctcattggatgaatgattgcgccctggcggtggtccatagcagcttccctggtctgtgtcaaggtgggccgatctcacaacataaaacataacagctccccctccttccaactgtttgttgatcttaatcaacttccccctttctttcaacttctctccttcctcccctccttctccctccctcctccaactctctccttcaccaaatctatcacatcctctttcctactttttttatgttatcctccataaatctctcatttgttgacatcctatacctttcctcaccccacacttaccgtttacgtttcgttcagtattcgttctctttcttaggccaccttctcttagatctctacccttacacttatcatagaactcttagtctttcccttctcctcccttaatctcctcttaacattcatcaac

SEQ ID NO: 8 - DNA, 1014 bp, synthetic construct
  misc_feature 1..1014: note = Synthetic constitutive promoter
  misc_feature 1..1014: note = Synthetic constitutive promoter BBa_K3046008|PLEAPhfbD_1|high
  source 1..1014: mol_type = other DNA
actctacgagtaggctagcattctaagcctcagagattcagtatccgcgccagagcgggacggccatctgcaaggggtaagacgcaccccgctggggtgggaatgtagcgaacttttgttatcatgttctcgcataatgcccttgtttaaaatgattcggtatgactgacatagagcctagtagtgaggaagtgtacttggcgagacaagggtactggcgaatcggcaggtagcgatagtttctgggaatgactataggtatgcaaaagactcgccaaacatggacgtttcctgatttcagcgcatgttatgacgcaatgctcaagccgattacgttatggaagatgagatgccatgctacattgattgtgatcagtttggtgaaatcaataccattacaagcagcatgatgcgaggcttgatgtgggttcatgaagatctttgtcctttatcttacggttcttcaaaggcataatgcgggatagcaatggacgggtctttgttggcctggagtagagcgagatttgggaggtagcaaaaggtatcgtttacgaatagagctctgtgggtcatcctgcatgaagaaccattcagctcaagcaatttcgacctagtccattgtcttaaaagtctccgggttatcttgaagatgagccaattgacaaaatacactgtgctagccgacgcagttctgggctgcaccgagtgacatgttgcgtgctttgtcctctacataaagcttgccattggtgagaggccagagggtcaatcacgttacaggatcaatatcttgtctcaagtatgcaaataggacgaataactgatataccaagtcaagtggcttataagccccaaataggacagtctccatgggcgagagagctatataaaccatcaaaaacccctatctttctactgcattttttcctcatcacaacacaattcctgtatcttatcattttcaaaagcaatactacacttcttctcaggcttacaaagaactcaatctatcac